European Patent Application EP 4 253 404 A2, published October 4, 2023. Title: New conjugates of montelukast and peptides. Applicant: EnliTISA (Shanghai) Pharmaceutical Co., Ltd. The sequence listing filed with the application follows.

SEQUENCE LISTING (48 sequences)

SEQ ID NO: 1 - protein, 37 aa, Hyalophora cecropia
  MOD_RES 1: note = Lysine residue with N-terminal hydrogen
  REGION 1..37: note = Cecropin A
  MOD_RES 37: note = Lysine residue with C-terminal carboxamide
XWKLFKKIEKVGQNIRDGIIKAGPAVAVVGQATQIAX

SEQ ID NO: 2 - protein, 35 aa, Hyalophora cecropia
  MOD_RES 1: note = Lysine residue with N-terminal hydrogen
  REGION 1..35: note = Cecropin B
  MOD_RES 35: note = Lysine residue with C-terminal carboxamide
XWKVFKKIEKMGRNIRNGIVKAGPAIAVLGEAKAX

SEQ ID NO: 3 - protein, 37 aa, Homo sapiens
  MOD_RES 1: note = Lysine residue with N-terminal hydrogen
  REGION 1..37: note = LL-37
  MOD_RES 37: note = Lysine residue with C-terminal carboxamide
XLGDFFRKSKEKIGKEFKRIVQRIKDFLRNLVPRTEX

SEQ ID NO: 4 - protein, 10 aa, synthetic construct
  SITE 6..7: note = Wherein X is 3- or 4-hydroxyproline
  SITE 9: note = Wherein X is 3,4-dihydroxyphenylalanine
AKPSYXXTXK

SEQ ID NO: 5 - skipped

SEQ ID NO: 6 - protein, 6 aa, synthetic construct
  SITE 4..5: note = Wherein X is 3- or 4-hydroxyproline
APSXXT

SEQ ID NO: 7-8 - skipped (2 entries)

SEQ ID NO: 9 - protein, 10 aa, synthetic construct
  SITE 4: note = Wherein X is serine or phosphoserine
  SITE 5: note = Wherein X is selected from the group consisting of 3,4-dihydroxyphenylalanine, tyrosine and phosphotyrosine
  SITE 6..7: note = Wherein X is 3- or 4-hydroxyproline
  VARIANT 9: note = Wherein X is tyrosine, phosphotyrosine, 3-hydroxyproline, 4-hydroxyproline, threonine, phosphothreonine or 3,4-dihydroxyphenylalanine
AKPXXXXTXK

SEQ ID NO: 10 - protein, 10 aa, synthetic construct
  SITE 4: note = Wherein X is serine or phosphoserine
  SITE 5: note = Wherein X is selected from the group consisting of 3,4-dihydroxyphenylalanine, tyrosine and phosphotyrosine
  SITE 6: note = Wherein X is 3- or 4-hydroxyproline
  VARIANT 8: note = Wherein X is tyrosine, phosphotyrosine, 3-hydroxyproline, 4-hydroxyproline, threonine, phosphothreonine or 3,4-dihydroxyphenylalanine
  SITE 9: note = Wherein X is 3- or 4-hydroxyproline
AKPXXXTXXK

SEQ ID NO: 11 - protein, 10 aa, synthetic construct
  SITE 4: note = Wherein X is phosphoserine
  SITE 6..7: note = Wherein X is 3- or 4-hydroxyproline
  SITE 9: note = Wherein X is 3,4-dihydroxyphenylalanine
AKPXYXXTXK

SEQ ID NO: 12 - protein, 10 aa, synthetic construct
  SITE 6..7: note = Wherein X is 3- or 4-hydroxyproline
AKPSYXXTYK

SEQ ID NO: 13 - protein, 10 aa, synthetic construct
  SITE 4: note = Wherein X is phosphoserine
  SITE 6..7: note = Wherein X is 3- or 4-hydroxyproline
AKPXYXXTYK

SEQ ID NO: 14 - protein, 7 aa, synthetic construct
  SITE 5: note = Wherein X is 3- or 4-hydroxyproline
  SITE 6: note = Wherein X is 3,4-dihydroxyphenylalanine
KPSYXXK

SEQ ID NO: 15 - protein, 7 aa, synthetic construct
  SITE 4: note = Wherein X is phosphotyrosine
  SITE 5: note = Wherein X is 3- or 4-hydroxyproline
  SITE 6: note = Wherein X is 3,4-dihydroxyphenylalanine
KPSXXXK

SEQ ID NO: 16 - protein, 10 aa, synthetic construct
  SITE 6..7: note = Wherein X is 3- or 4-hydroxyproline
  SITE 8: note = Wherein X is phosphothreonine
  SITE 9: note = Wherein X is 3,4-dihydroxyphenylalanine
AKPSYXXXXK

SEQ ID NO: 17 - protein, 10 aa, synthetic construct
  SITE 6..7: note = Wherein X is 3- or 4-hydroxyproline
  SITE 8: note = Wherein X is phosphothreonine
AKPSYXXXYK

SEQ ID NO: 18 - protein, 11 aa, synthetic construct
  SITE 6..7: note = Wherein X is 3- or 4-hydroxyproline
  SITE 9: note = Wherein Xaa is 3,4-dihydroxyphenylalanine
  SITE 10: note = Wherein X is 3- or 4-hydroxyproline
AKPSYXXTXXK

SEQ ID NO: 19 - protein, 11 aa, synthetic construct
  SITE 4: note = Wherein X is phosphoserine
  SITE 6..7: note = Wherein X is 3- or 4-hydroxyproline
  SITE 9: note = Wherein X is 3,4-dihydroxyphenylalanine
  SITE 10: note = Wherein X is 3- or 4-hydroxyproline
AKPXYXXTXXK

SEQ ID NO: 20 - protein, 11 aa, synthetic construct
  SITE 6..7: note = Wherein X is 3- or 4-hydroxyproline
  SITE 10: note = Wherein X is 3- or 4-hydroxyproline
AKPSYXXTYXK

SEQ ID NO: 21 - protein, 11 aa, synthetic construct
  SITE 4: note = Wherein X is phosphoserine
  SITE 6..7: note = Wherein X is 3- or 4-hydroxyproline
  SITE 10: note = Wherein X is 3- or 4-hydroxyproline
AKPXYXXTYXK

SEQ ID NO: 22 - protein, 10 aa, synthetic construct
  SITE 6: note = Wherein X is 3- or 4-hydroxyproline
  SITE 8: note = Wherein Xaa is 3,4-dihydroxyphenylalanine
  SITE 9: note = Wherein X is 3- or 4-hydroxyproline
AKPSYXTXXK

SEQ ID NO: 23 - protein, 9 aa, synthetic construct
  SITE 4: note = Wherein X is phosphoserine
  SITE 6: note = Wherein X is 3- or 4-hydroxyproline
  SITE 8: note = Wherein X is 3,4-dihydroxyphenylalanine
  SITE 9: note = Wherein X is 3- or 4-hydroxyproline
AKPXYXTXK

SEQ ID NO: 24 - protein, 10 aa, synthetic construct
  SITE 6: note = Wherein X is 3- or 4-hydroxyproline
  SITE 9: note = Wherein X is 3- or 4-hydroxyproline
AKPSYXTYXK

SEQ ID NO: 25 - protein, 10 aa, synthetic construct
  SITE 4: note = Wherein X is phosphoserine
  SITE 6: note = Wherein X is 3- or 4-hydroxyproline
  SITE 9: note = Wherein X is 3- or 4-hydroxyproline
AKPXYXTYXK

SEQ ID NO: 26 - protein, 11 aa, synthetic construct
  SITE 6..7: note = Wherein X is 3- or 4-hydroxyproline
  SITE 8: note = Wherein X is phosphothreonine
  SITE 9: note = Wherein X is 3,4-dihydroxyphenylalanine
  SITE 10: note = Wherein X is 3- or 4-hydroxyproline
AKPSYXXXXXK

SEQ ID NO: 27 - protein, 11 aa, synthetic construct
  SITE 6..7: note = Wherein X is 3- or 4-hydroxyproline
  SITE 8: note = Wherein X is phosphothreonine
  SITE 10: note = Wherein X is 3- or 4-hydroxyproline
AKPSYXXXYXK

SEQ ID NO: 28 - protein, 9 aa, synthetic construct
  SITE 6..7: note = Wherein X is 3- or 4-hydroxyproline
  SITE 9: note = Wherein X is 3,4-dihydroxyphenylalanine
AKPSYXXTX

SEQ ID NO: 29 - protein, 9 aa, synthetic construct
  SITE 4: note = Wherein X is phosphoserine
  SITE 6..7: note = Wherein X is 3- or 4-hydroxyproline
  SITE 9: note = Wherein X is 3,4-dihydroxyphenylalanine
AKPXYXXTX

SEQ ID NO: 30 - protein, 9 aa, synthetic construct
  SITE 6..7: note = Wherein X is 3- or 4-hydroxyproline
AKPSYXXTY

SEQ ID NO: 31 - protein, 9 aa, synthetic construct
  SITE 4: note = Wherein X is phosphoserine
  SITE 6..7: note = Wherein X is 3- or 4-hydroxyproline
AKPXYXXTY

SEQ ID NO: 32 - protein, 6 aa, synthetic construct
  SITE 5: note = Wherein X is 3- or 4-hydroxyproline
  SITE 6: note = Wherein X is 3,4-dihydroxyphenylalanine
KPSYXX

SEQ ID NO: 33 - skipped

SEQ ID NO: 34 - protein, 9 aa, synthetic construct
  SITE 6..7: note = Wherein X is 3- or 4-hydroxyproline
  SITE 8: note = Wherein X is phosphothreonine
  SITE 9: note = Wherein X is 3,4-dihydroxyphenylalanine
AKPSYXXXX

SEQ ID NO: 35 - protein, 9 aa, synthetic construct
  SITE 6..7: note = Wherein X is 3- or 4-hydroxyproline
  SITE 8: note = Wherein X is phosphothreonine
AKPSYXXXY

SEQ ID NO: 36 - protein, 10 aa, synthetic construct
  SITE 6..7: note = Wherein X is 3- or 4-hydroxyproline
  SITE 9: note = Wherein X is 3,4-dihydroxyphenylalanine
  SITE 10: note = Wherein X is 3- or 4-hydroxyproline
AKPSYXXTXX

SEQ ID NO: 37 - protein, 10 aa, synthetic construct
  SITE 4: note = Wherein X is phosphoserine
  SITE 6..7: note = Wherein X is 3- or 4-hydroxyproline
  SITE 9: note = Wherein X is 3,4-dihydroxyphenylalanine
  SITE 10: note = Wherein X is 3- or 4-hydroxyproline
AKPXYXXTXX

SEQ ID NO: 38 - protein, 10 aa, synthetic construct
  SITE 6..7: note = Wherein X is 3- or 4-hydroxyproline
  SITE 10: note = Wherein X is 3- or 4-hydroxyproline
AKPSYXXTYX

SEQ ID NO: 39 - protein, 10 aa, synthetic construct
  SITE 4: note = Wherein X is phosphoserine
  SITE 6..7: note = Wherein X is 3- or 4-hydroxyproline
  SITE 10: note = Wherein X is 3- or 4-hydroxyproline
AKPXYXXTYX

SEQ ID NO: 40 - protein, 9 aa, synthetic construct
  SITE 6: note = Wherein X is 3- or 4-hydroxyproline
  SITE 8: note = Wherein X is 3,4-dihydroxyphenylalanine
  SITE 9: note = Wherein X is 3- or 4-hydroxyproline
AKPSYXTXX

SEQ ID NO: 41 - protein, 9 aa, synthetic construct
  SITE 4: note = Wherein X is phosphoserine
  SITE 6: note = Wherein X is 3- or 4-hydroxyproline
  SITE 8: note = Wherein X is 3,4-dihydroxyphenylalanine
  SITE 9: note = Wherein X is 3- or 4-hydroxyproline
AKPXYXTXX

SEQ ID NO: 42 - protein, 9 aa, synthetic construct
  SITE 6: note = Wherein X is 3- or 4-hydroxyproline
  SITE 9: note = Wherein X is 3- or 4-hydroxyproline
AKPSYXTYX

SEQ ID NO: 43 - protein, 9 aa, synthetic construct
  SITE 4: note = Wherein X is phosphoserine
  SITE 6: note = Wherein X is 3- or 4-hydroxyproline
  SITE 9: note = Wherein X is 3- or 4-hydroxyproline
AKPXYXTYX

SEQ ID NO: 44 - protein, 10 aa, synthetic construct
  SITE 6..7: note = Wherein X is 3- or 4-hydroxyproline
  SITE 8: note = Wherein X is phosphothreonine
  SITE 9: note = Wherein X is 3,4-dihydroxyphenylalanine
  SITE 10: note = Wherein X is 3- or 4-hydroxyproline
AKPSYXXXXX

SEQ ID NO: 45 - protein, 10 aa, synthetic construct
  SITE 6..7: note = Wherein X is 3- or 4-hydroxyproline
  SITE 8: note = Wherein X is phosphothreonine
  SITE 10: note = Wherein X is 3- or 4-hydroxyproline
AKPSYXXXYX

SEQ ID NO: 46 - protein, 7 aa, synthetic construct
  SITE 6..7: note = Wherein X is 3- or 4-hydroxyproline
AKPSYXX

SEQ ID NO: 47 - protein, 6 aa, synthetic construct
  SITE 6: note = Wherein X is 3- or 4-hydroxyproline
AKPSYX

SEQ ID NO: 48 - skipped